European Patent Specification EP 3 729 096 B1, published July 15, 2026. Title: SPARC Assay. Applicant: Nordic Bioscience A/S. The sequence listing filed with the application follows.

SEQUENCE LISTING (11 sequences)

SEQ ID NO: 1 - protein, 10 aa, Artificial Sequence
  N-terminus biomarker
LLARDFEKNY

SEQ ID NO: 2 - protein, 11 aa, Artificial Sequence
  Elongated peptide
ELLARDFEKNY

SEQ ID NO: 3 - protein, 9 aa, Artificial Sequence
  Truncated peptide
LARDFEKNY

SEQ ID NO: 4 - protein, 10 aa, Artificial Sequence
  nonsense peptide
VPKDLPPDTT

SEQ ID NO: 5 - protein, 10 aa, Artificial Sequence
  nonsense coating peptide
  SITE 10: C-terminal biotinylated
VPKDLPPDTT

SEQ ID NO: 6 - protein, 13 aa, Artificial Sequence
  Immunogenic peptide
  SITE 13: KLH attached to C-terminus
LLARDFEKNYGGC

SEQ ID NO: 7 - protein, 11 aa, Artificial Sequence
  Biotinylated coating peptide
  SITE 11: C-terminal biotinylated
LLARDFEKNYK

SEQ ID NO: 8 - protein, 10 aa, Artificial Sequence
  Von Willebrand factor
LLARDCQDHS

SEQ ID NO: 9 - protein, 10 aa, Artificial Sequence
  GCG
LAARDFINWL

SEQ ID NO: 10 - protein, 10 aa, Artificial Sequence
  SPARC-like protein 1
LLLRDFKKNY

SEQ ID NO: 11 - protein, 10 aa, Artificial Sequence
  ADAMTS15
LLARDQCNLH